European Patent Application EP 4 365 187 A1, published May 8, 2024. Title: PEPTIDES HAVING ANCANCER ACTIVITY AND USES THEREOF. Applicant: Korea University Research and Business Foundation. The sequence listing filed with the application follows.

SEQUENCE LISTING (5 sequences)

SEQ ID NO: 1 - protein, 10 aa, Mus musculus
EKAEEDRYFR

SEQ ID NO: 2 - protein, 10 aa, Homo sapiens
EQAEEERYFR

SEQ ID NO: 3 - protein, 3 aa, Homo sapiens
YFR

SEQ ID NO: 4 - protein, 7 aa, Homo sapiens
EQAEEER

SEQ ID NO: 5 - protein, 12 aa, Homo sapiens
AQSREQLAALKK